European Patent Specification EP 3 987 051 B1, published May 20, 2026. Title: RATIOMETRIC DETECTION OF LUCIFERASE ASSAYS USING A CALIBRATOR LUCIFERASE. Applicant: Technische Universiteit Eindhoven. The sequence listing filed with the application follows.

SEQUENCE LISTING (6 sequences)

SEQ ID NO: 1 - protein, 11 aa, Oplophorus gracilirostris
  SBiT with K(d) of 190 µM
VTGYRLFEEIL

SEQ ID NO: 2 - protein, 11 aa, Oplophorus gracilirostris
  SBiT with K(d) of 0.28 µM
VTGYRLFEKIL

SEQ ID NO: 3 - DNA, 507 bp, Artificial Sequence
  DNA sequence of pG-SB
atgggctggagccatccgcagtttgaaaaaggtggtagcatgacatttaaactgattatcaacggcaaaactttaaagggagagatcacaatagaagcggtggatgcttaggaggcggagaagatttttaagcagtatgcaaatgattatggaattgatggtgaatggacttatgacgacgcaactaaaactttcacggtaacagaagaatttacaggaggttcgggtgggtcgggaggttctggcggctctggaggaagtggtggtagcggtgaattcgccgaagcagccgctaaagaagccgcagcaaaggaagccgcggccaaggaggcagccgcaaaagaggccgcggcgaaggaagcagcagccaaggcagaattcgggggtagcggcggctcggggggtagtggtggaagcgggggttcaggcggttctgggggtaccgttaccggctatcgtctgtttgaaaaagagagcggcggttcacatcatcatcaccaccattaa

SEQ ID NO: 4 - DNA, 948 bp, Artificial Sequence
  DNA sequence of pG-LB
atgggctggagccatccgcagtttgaaaaaggtggtagcatgacatttaaactgattatcaacggcaaaactttaaagggagagatcacaatagaagcggtggatgcttaggaggcggagaagatttttaagcagtatgcaaatgattatggaattgatggtgaatggacttatgacgacgcaactaaaactttcacggtaacagaagaatttacaggaggttcgggtgggtcgggaggttctggcggctctggaggaagtggtggtagcggtgaattcgccgaagcagccgctaaagaagccgcagcaaaggaagccgcggccaaggaggcagccgcaaaagaggccgcggcgaaggaagcagcagccaaggcagaattcgggggtagcggcggctcggggggtagtggtggaagcgggggttcaggcggttctgggggtaccgtcttcacactcgaagatttcgttggggactgggaacagacagccgcctacaacctggaccaagtccttgaacagggaggtgtgtccagtttgctgcagaatctcgccgtgtccgtaactccgatccaaaggattgtccggagcggtgaaaatgccctgaagatcgacatccatgtcatcatcccgtatgaaggtctgagcgccgaccaaatggcccagatcgaagaggtgtttaaggtggtgtaccctgtggatgatcatcactttaaggtgatcctgccctatggcacactggtaatcgacggggttacgccgaacatgctgaactatttcggacggccgtatgaaggcatcgccgtgttcgacggcaaaaagatcactgtaacagggaccctgtggaacggcaacaaaattatcgacgagcgcctgatcacccccgacggctccatgctgttccgagtaaccatcaacagcggaggttcccaccaccaccatcaccactaa

SEQ ID NO: 5 - DNA, 594 bp, Artificial Sequence
  DNA sequence of K9C/D157C/G191C variant
atgtggtctcatcctcaatttgaatgcatggtatttactcttgaagattttgtcggtgattggcgccagaccgccggctataacctggaccaagtgcttgaacagggcggggttagcagcctgtttcaaaacctgggggtgagtgtcacgccaattcagcgcatcgttctgtcgggagagaatggtctgaaaatcgatatccacgtcattatcccgtacgaaggtctttctggtgatcagatggggcagatagaaaaaatattcaaagtggtgtacccagtagacgatcatcacttcaaggttatactgcactatggcaccctcgttatcgatggcgttactccgaatatgatcgattactttgggcgtccttatgaaggtattgcggtgttcgacggtaaaaaaattacggttaccgggacgctctggaatggtaataaaatcattgatgagcgcttgataaacccatgtggcagccttctgttcagagttacgataaacggggttacgggttggcgactgagcgaaagaatattagctgcgtccgcactcgagctgccagaaaccggttgtcaccaccaccaccaccactga

SEQ ID NO: 6 - DNA, 1149 bp, Artificial Sequence
  DNA sequence of TNFa-SB
atgtcggactcagaagtcaatcaagaagctaagccagaggtcaagccagaagtcaagcctgagactcacatcaatttaaaggtgtccgatggatcttcagagatcttcttcaagatcaaaaagaccactcctttaagaaggctgatggaagcgttcgctaaaagacagggtaaggaaatggactccttaagattcttgtacgacggtattagaattcaagctgatcagacccctgaagatttggacatggaggataacgatattattgaggctcacagagaacagattggtggtgtgcgtagcagcagccgtaccccgagcgataaaccggtggcgcatgtggtggcgaatccgcaggcggaaggccagctgcagtggctgaaccgtcgtgcgaatgcgctgctggccaacggcgtggaactgcgtgataatcagctggttgtgccgagcgaaggcctgtatctgatttatagccaggtgctgtttaaaggccagggctgcccgagcacccatgtgctgctgacccataccattagccgtattgcggtgagctatcagaccaaagtgaacctgctgtctgcgattaaaagcccgtgccagcgtgaaaccccggaaggcgcggaagcgaaaccgtggtatgaaccgatttatctgggcggcgtgtttcagctggaaaaaggcgatcgtctgagcgcggaaattaaccgtccggattatctggattttgcggaaagcggccaggtgtattttggcattattgcgctgggatccggggggagcggtggtagcggtgggtccgggggaagtggtggcagtggtgggtccggagggagtggcgggtcgggaggaagcgggggctcaggatccgggggcagtggcggctcaggaggttctggaggctcaggcggaagcgggggtagcgaagcagccgcaaaagaagcagccgccaaggaagcagcagcaaaggaggcagctgcaaaggaggcggcggcgaaagaggcggcagccaaaggaggatctggtggctcaggtggtagtggaggatcaggaggtagtggcggatcaggtaccgttaccggctatcgtctgtttgaaaaagagagcggtggttcagggggctcgtggtcacatccgcaatttgaaaagtaa